European Patent Application EP 4 180 525 A1, published May 17, 2023. Title: MODIFIED L-ASPARAGINASE. Applicant: Jazz Pharmaceuticals Ireland Limited. Application EP. The sequence listing filed with the application follows.

SEQUENCE LISTING (17 sequences)

SEQ ID NO: 1 - protein, 327 aa, Dickeya chrysanthemi
  REGION 1..327: note = L-Asparaginase
ADKLPNIVILATGGTIAGSAATGTQTTGYKAGALGVDTLINAVPEVKKLANVKGEQFSNMASENMTGDVVLKLSQRVNELLARDDVDGVVITHGTDTVEESAYFLHLTVKSDKPVVFVAAMRPATAISADGPMNLLEAVRVAGDKQSRGRGVMVVLNDRIGSARYITKTNASTLDTFKANEEGYLGVIIGNRIYYQNRIDKLHTTRSVFDVRGLTSLPKVDILYGYQDDPEYLYDAAIQHGVKGIVYAGMGAGSVSVRGIAGMRKAMEKGVVVIRSTRTGNGIVPPDEELPGLVSDSLNPAHARILLMLALTRTSDPKVIQEYFHTY

SEQ ID NO: 2 - DNA, 981 bp, Dickeya chrysanthemi
  misc_feature 1..981: note = L-Asparaginase
  source 1..981: mol_type = other DNA
gcagataaactgccgaatattgttattctggcaaccggtggcaccattgcaggtagcgcagcaaccggcacccaaaccacaggttataaagccggtgcactgggtgttgataccctgattaatgcagttccggaagttaaaaaactggccaatgtgaaaggtgaacagtttagcaatatggccagcgaaaatatgaccggtgatgttgttctgaaactgagccagcgtgttaatgaactgctggcacgtgatgatgttgatggtgtggttattacccatggcaccgataccgttgaagaaagcgcctattttctgcatctgaccgtgaaaagcgataaaccggttgtttttgttgcagcaatgcgtccggcaaccgcaattagcgcagatggtccgatgaatctgctggaagcagttcgtgttgccggtgataaacagagccgtggtcgtggtgttatggttgttctgaatgatcgtattggtagcgcacgctatattaccaaaaccaatgcaagcaccctggatacctttaaagccaatgaagaaggttatctgggcgttattattggcaatcgcatttattatcagaatcgcattgataaactgcataccacccgtagcgtttttgatgttcgtggtctgaccagcctgccgaaagttgatattctgtatggctatcaggatgatccggaatatctgtatgatgcagccattcagcatggtgttaaaggtattgtgtatgcaggtatgggtgcaggtagcgttagcgttcgtggtattgcaggtatgcgtaaagcaatggaaaaaggcgttgttgttattcgtagcacccgtaccggtaatggtattgttccgccggatgaagaactgccgggtctggttagcgatagcctgaatccggcacatgcacgtattctgctgatgctggcactgacccgtaccagcgatccgaaagtgattcaggaatattttcatacctat

SEQ ID NO: 3 - protein, 366 aa, Dickeya chrysanthemi
  REGION 1..366: note = L-Asparaginase with signal peptide
MFKFKKNFLVGLSAALMSISLFSATASAARRAIVGRSSAADKLPNIVILATGGTIAGSAATGTQTTGYKAGALGVDTLINAVPEVKKLANVKGEQFSNMASENMTGDVVLKLSQRVNELLARDDVDGVVITHGTDTVEESAYFLHLTVKSDKPVVFVAAMRPATAISADGPMNLLEAVRVAGDKQSRGRGVMVVLNDRIGSARYITKTNASTLDTFKANEEGYLGVIIGNRIYYQNRIDKLHTTRSVFDVRGLTSLPKVDILYGYQDDPEYLYDAAIQHGVKGIVYAGMGAGSVSVRGIAGMRKAMEKGVVVIRSTRTGNGIVPPDEELPGLVSDSLNPAHARILLMLALTRTSDPKVIQEYFHTY

SEQ ID NO: 4 - DNA, 1147 bp, Dickeya chrysanthemi
  misc_feature 1..1147: note = L-Asparaginase
  source 1..1147: mol_type = other DNA
tctagaaataattttgtttaactttaagaaggagatatacatatgttcaaattcaaaaaaaacttcctggtgggtctgagcgcagcactgatgagcattagcctgtttagcgcaaccgcaagcgcagccagaagagcgattgtaggacgctcttctgccgcagataaactgccgaatattgttattctggcaaccggtggcaccattgcaggtagcgcagcaaccggcacccagaccaccggttataaagccggtgcactgggtgttgataccctgattaatgcagttccggaagttaaaaaactggccaatgttaaaggtgagcagtttagcaatatggccagcgaaaatatgaccggtgatgttgttctgaaactgagccagcgtgttaatgaactgctggcacgtgatgatgttgatggtgttgttattacccatggcaccgataccgttgaagaaagcgcatattttctgcatctgaccgtgaaaagcgataaaccggttgtttttgttgcagcaatgcgtccggcaaccgccattagcgcagatggtccgatgaatctgctggaagcagttcgtgttgccggtgataaacagagccgtggtcgtggtgttatggttgtgctgaatgatcgtattggtagcgcacgttatattaccaaaaccaatgcaagcaccctggatacctttaaagcaaatgaagaaggttatctgggcgtcattattggcaatcgtatctattatcagaaccgcatcgacaaactgcataccacccgtagcgtttttgatgttcgtggtctgaccagcctgccgaaagtggatattctgtatggttatcaggatgatccggaatatctgtatgatgcagcaattcagcatggtgtgaaaggtattgtttatgcaggtatgggtgcgggtagcgttagcgttcgtggtattgccggtatgcgtaaagcaatggaaaaaggtgttgttgtgattcgtagcacccgtaccggtaatggtattgttccgcctgatgaagaactgcctggtctggttagcgatagcctgaatccggcacatgcacgtattctgctgatgctggcactgacccgtaccagcgatccgaaagttattcaagaatattttcatacctattaagctt

SEQ ID NO: 5 - protein, 20 aa, Synthetic construct
  REGION 1..20: note = PA(20) peptide
AAPAAPAPAAPAAPAPAAPA

SEQ ID NO: 6 - DNA, 60 bp, Synthetic construct
  misc_feature 1..60: note = PA(20) peptide
  source 1..60: mol_type = other DNA
gccgcgccagcggccccggcccctgccgcgcccgctgctcccgcccctgctgccccagcc

SEQ ID NO: 7 - protein, 201 aa, Synthetic construct
  REGION 1..201: note = PA(200)-polypeptide
AAPAAPAPAAPAAPAPAAPAAAPAAPAPAAPAAPAPAAPAAAPAAPAPAAPAAPAPAAPAAAPAAPAPAAPAAPAPAAPAAAPAAPAPAAPAAPAPAAPAAAPAAPAPAAPAAPAPAAPAAAPAAPAPAAPAAPAPAAPAAAPAAPAPAAPAAPAPAAPAAAPAAPAPAAPAAPAPAAPAAAPAAPAPAAPAAPAPAAPAA

SEQ ID NO: 8 - DNA, 603 bp, Synthetic construct
  misc_feature 1..603: note = PA(200)-polypeptide
  source 1..603: mol_type = other DNA
gccgcgccagcggccccggcccctgccgcgcccgctgctcccgcccctgctgccccagccgccgctcctgcggcacctgcgcccgccgcgccggcagcgccggcaccggcagctccggcggccgcgcctgcagctcctgcaccggcggctccagcagccccggcgccggccgcacctgcggcggcgcccgcggcgcctgcacccgcagcgcctgcggcaccggccccagcagcccctgccgccgcaccggctgcgcctgccccagcggcccccgctgccccggccccggcggctccagccgcagcgcctgccgccccagcgcccgcagcaccggcggcaccagctccggcggcgccggcggcggctccggcagctccggcccctgctgcgccggctgcgccggctccggcggcccctgcggcggctccggccgcacctgcacctgccgcgccggctgctccggccccggctgccccagcagcggcaccagcagcgcctgctcctgcggcgcctgcagctccggcgccggcagccccggccgccgcacccgcggctccagcccccgccgctccagcagcccccgcgccagctgcacctgctgcc

SEQ ID NO: 9 - protein, 401 aa, Synthetic construct
  REGION 1..401: note = PA(400)-polypeptide
AAPAAPAPAAPAAPAPAAPAAAPAAPAPAAPAAPAPAAPAAAPAAPAPAAPAAPAPAAPAAAPAAPAPAAPAAPAPAAPAAAPAAPAPAAPAAPAPAAPAAAPAAPAPAAPAAPAPAAPAAAPAAPAPAAPAAPAPAAPAAAPAAPAPAAPAAPAPAAPAAAPAAPAPAAPAAPAPAAPAAAPAAPAPAAPAAPAPAAPAAAPAAPAPAAPAAPAPAAPAAAPAAPAPAAPAAPAPAAPAAAPAAPAPAAPAAPAPAAPAAAPAAPAPAAPAAPAPAAPAAAPAAPAPAAPAAPAPAAPAAAPAAPAPAAPAAPAPAAPAAAPAAPAPAAPAAPAPAAPAAAPAAPAPAAPAAPAPAAPAAAPAAPAPAAPAAPAPAAPAAAPAAPAPAAPAAPAPAAPAA

SEQ ID NO: 10 - DNA, 1203 bp, Synthetic construct
  misc_feature 1..1203: note = PA(400)-polypeptide
  source 1..1203: mol_type = other DNA
gccgcgccagcggccccggcccctgccgcgcccgctgctcccgcccctgctgccccagccgccgctcctgcggcacctgcgcccgccgcgccggcagcgccggcaccggcagctccggcggccgcgcctgcagctcctgcaccggcggctccagcagccccggcgccggccgcacctgcggcggcgcccgcggcgcctgcacccgcagcgcctgcggcaccggccccagcagcccctgccgccgcaccggctgcgcctgccccagcggcccccgctgccccggccccggcggctccagccgcagcgcctgccgccccagcgcccgcagcaccggcggcaccagctccggcggcgccggcggcggctccggcagctccggcccctgctgcgccggctgcgccggctccggcggcccctgcggcggctccggccgcacctgcacctgccgcgccggctgctccggccccggctgccccagcagcggcaccagcagcgcctgctcctgcggcgcctgcagctccggcgccggcagccccggccgccgcacccgcggctccagcccccgccgctccagcagcccccgcgccagctgcacctgctgccgctcctgctgcccctgctcccgctgcccccgccgcccccgccccagctgcccccgctgccgcacctgctgccccagctcccgctgccccagccgcgccggcccccgcagctccagccgcggcaccagctgccccagctccagcggcgcctgctgccccggcccccgcggcaccggctgccgcgcccgcagctccagcgcctgctgcaccggctgctccggcacccgccgcgccagcagctgcccctgcggcaccagctcctgctgcccccgcggcacctgcacccgctgccccggcggcagctcccgccgcgccagcccctgcagctcctgctgcacctgctcctgccgcccctgctgctgcccctgctgctccagcccctgcagcaccggccgctccagctcctgccgctcctgccgctgcgcccgctgctccagccccagctgcgccagcagctcctgcacctgctgcccctgccgccgcccctgcggctccagcacctgctgcaccggccgccccggcgcccgctgcccccgcagcagccccagccgcacccgctccagcagctcccgcagccccagcacccgcagcaccagccgcc

SEQ ID NO: 11 - protein, 528 aa, Synthetic construct
  REGION 1..528: note = Asparaginase-PA(200)-fusion protein
AAPAAPAPAAPAAPAPAAPAAAPAAPAPAAPAAPAPAAPAAAPAAPAPAAPAAPAPAAPAAAPAAPAPAAPAAPAPAAPAAAPAAPAPAAPAAPAPAAPAAAPAAPAPAAPAAPAPAAPAAAPAAPAPAAPAAPAPAAPAAAPAAPAPAAPAAPAPAAPAAAPAAPAPAAPAAPAPAAPAAAPAAPAPAAPAAPAPAAPAAADKLPNIVILATGGTIAGSAATGTQTTGYKAGALGVDTLINAVPEVKKLANVKGEQFSNMASENMTGDVVLKLSQRVNELLARDDVDGVVITHGTDTVEESAYFLHLTVKSDKPVVFVAAMRPATAISADGPMNLLEAVRVAGDKQSRGRGVMVVLNDRIGSARYITKTNASTLDTFKANEEGYLGVIIGNRIYYQNRIDKLHTTRSVFDVRGLTSLPKVDILYGYQDDPEYLYDAAIQHGVKGIVYAGMGAGSVSVRGIAGMRKAMEKGVVVIRSTRTGNGIVPPDEELPGLVSDSLNPAHARILLMLALTRTSDPKVIQEYFHTY

SEQ ID NO: 12 - DNA, 1717 bp, Synthetic construct
  misc_feature 1..1717: note = Asparaginase-PA(200)-fusion protein
  source 1..1717: mol_type = other DNA
tctagaaataattttgtttaactttaagaaggagatatacatatgttcaaattcaaaaaaaacttcctggtgggtctgagcgcagcactgatgagcattagcctgtttagcgcaaccgcaagcgcagccgcgccagcggccccggcccctgccgcgcccgctgctcccgcccctgctgccccagccgccgctcctgcggcacctgcgcccgccgcgccggcagcgccggcaccggcagctccggcggccgcgcctgcagctcctgcaccggcggctccagcagccccggcgccggccgcacctgcggcggcgcccgcggcgcctgcacccgcagcgcctgcggcaccggccccagcagcccctgccgccgcaccggctgcgcctgccccagcggcccccgctgccccggccccggcggctccagccgcagcgcctgccgccccagcgcccgcagcaccggcggcaccagctccggcggcgccggcggcggctccggcagctccggcccctgctgcgccggctgcgccggctccggcggcccctgcggcggctccggccgcacctgcacctgccgcgccggctgctccggccccggctgccccagcagcggcaccagcagcgcctgctcctgcggcgcctgcagctccggcgccggcagccccggccgccgcacccgcggctccagcccccgccgctccagcagcccccgcgccagctgcacctgctgccgcagataaactgccgaatattgttattctggcaaccggtggcaccattgcaggtagcgcagcaaccggcacccagaccaccggttataaagccggtgcactgggtgttgataccctgattaatgcagttccggaagttaaaaaactggccaatgttaaaggtgagcagtttagcaatatggccagcgaaaatatgaccggtgatgttgttctgaaactgagccagcgtgttaatgaactgctggcacgtgatgatgttgatggtgttgttattacccatggcaccgataccgttgaagaaagcgcatattttctgcatctgaccgtgaaaagcgataaaccggttgtttttgttgcagcaatgcgtccggcaaccgccattagcgcagatggtccgatgaatctgctggaagcagttcgtgttgccggtgataaacagagccgtggtcgtggtgttatggttgtgctgaatgatcgtattggtagcgcacgttatattaccaaaaccaatgcaagcaccctggatacctttaaagcaaatgaagaaggttatctgggcgtcattattggcaatcgtatctattatcagaaccgcatcgacaaactgcataccacccgtagcgtttttgatgttcgtggtctgaccagcctgccgaaagtggatattctgtatggttatcaggatgatccggaatatctgtatgatgcagcaattcagcatggtgtgaaaggtattgtttatgcaggtatgggtgcgggtagcgttagcgttcgtggtattgccggtatgcgtaaagcaatggaaaaaggtgttgttgtgattcgtagcacccgtaccggtaatggtattgttccgcctgatgaagaactgcctggtctggttagcgatagcctgaatccggcacatgcacgtattctgctgatgctggcactgacccgtaccagcgatccgaaagttattcaagaatattttcatacctattaagctt

SEQ ID NO: 13 - protein, 728 aa, Synthetic construct
  REGION 1..728: note = Asparaginase-PA-(400)-fusion protein
AAPAAPAPAAPAAPAPAAPAAAPAAPAPAAPAAPAPAAPAAAPAAPAPAAPAAPAPAAPAAAPAAPAPAAPAAPAPAAPAAAPAAPAPAAPAAPAPAAPAAAPAAPAPAAPAAPAPAAPAAAPAAPAPAAPAAPAPAAPAAAPAAPAPAAPAAPAPAAPAAAPAAPAPAAPAAPAPAAPAAAPAAPAPAAPAAPAPAAPAAAPAAPAPAAPAAPAPAAPAAAPAAPAPAAPAAPAPAAPAAAPAAPAPAAPAAPAPAAPAAAPAAPAPAAPAAPAPAAPAAAPAAPAPAAPAAPAPAAPAAAPAAPAPAAPAAPAPAAPAAAPAAPAPAAPAAPAPAAPAAAPAAPAPAAPAAPAPAAPAAAPAAPAPAAPAAPAPAAPAAAPAAPAPAAPAAPAPAAPAAADKLPNIVILATGGTIAGSAATGTQTTGYKAGALGVDTLINAVPEVKKLANVKGEQFSNMASENMTGDVVLKLSQRVNELLARDDVDGVVITHGTDTVEESAYFLHLTVKSDKPVVFVAAMRPATAISADGPMNLLEAVRVAGDKQSRGRGVMVVLNDRIGSARYITKTNASTLDTFKANEEGYLGVIIGNRIYYQNRIDKLHTTRSVFDVRGLTSLPKVDILYGYQDDPEYLYDAAIQHGVKGIVYAGMGAGSVSVRGIAGMRKAMEKGVVVIRSTRTGNGIVPPDEELPGLVSDSLNPAHARILLMLALTRTSDPKVIQEYFHTY

SEQ ID NO: 14 - DNA, 2317 bp, Synthetic construct
  misc_feature 1..2317: note = Asparaginase-PA(400)-fusion protein
  source 1..2317: mol_type = other DNA
tctagaaataattttgtttaactttaagaaggagatatacatatgttcaaattcaaaaaaaacttcctggtgggtctgagcgcagcactgatgagcattagcctgtttagcgcaaccgcaagcgcagccgcgccagcggccccggcccctgccgcgcccgctgctcccgcccctgctgccccagccgccgctcctgcggcacctgcgcccgccgcgccggcagcgccggcaccggcagctccggcggccgcgcctgcagctcctgcaccggcggctccagcagccccggcgccggccgcacctgcggcggcgcccgcggcgcctgcacccgcagcgcctgcggcaccggccccagcagcccctgccgccgcaccggctgcgcctgccccagcggcccccgctgccccggccccggcggctccagccgcagcgcctgccgccccagcgcccgcagcaccggcggcaccagctccggcggcgccggcggcggctccggcagctccggcccctgctgcgccggctgcgccggctccggcggcccctgcggcggctccggccgcacctgcacctgccgcgccggctgctccggccccggctgccccagcagcggcaccagcagcgcctgctcctgcggcgcctgcagctccggcgccggcagccccggccgccgcacccgcggctccagcccccgccgctccagcagcccccgcgccagctgcacctgctgccgctcctgctgcccctgctcccgctgcccccgccgcccccgccccagctgcccccgctgccgcacctgctgccccagctcccgctgccccagccgcgccggcccccgcagctccagccgcggcaccagctgccccagctccagcggcgcctgctgccccggcccccgcggcaccggctgccgcgcccgcagctccagcgcctgctgcaccggctgctccggcacccgccgcgccagcagctgcccctgcggcaccagctcctgctgcccccgcggcacctgcacccgctgccccggcggcagctcccgccgcgccagcccctgcagctcctgctgcacctgctcctgccgcccctgctgctgcccctgctgctccagcccctgcagcaccggccgctccagctcctgccgctcctgccgctgcgcccgctgctccagccccagctgcgccagcagctcctgcacctgctgcccctgccgccgcccctgcggctccagcacctgctgcaccggccgccccggcgcccgctgcccccgcagcagccccagccgcacccgctccagcagctcccgcagccccagcacccgcagcaccagccgccgcagataaactgccgaatattgttattctggcaaccggtggcaccattgcaggtagcgcagcaaccggcacccagaccaccggttataaagccggtgcactgggtgttgataccctgattaatgcagttccggaagttaaaaaactggccaatgttaaaggtgagcagtttagcaatatggccagcgaaaatatgaccggtgatgttgttctgaaactgagccagcgtgttaatgaactgctggcacgtgatgatgttgatggtgttgttattacccatggcaccgataccgttgaagaaagcgcatattttctgcatctgaccgtgaaaagcgataaaccggttgtttttgttgcagcaatgcgtccggcaaccgccattagcgcagatggtccgatgaatctgctggaagcagttcgtgttgccggtgataaacagagccgtggtcgtggtgttatggttgtgctgaatgatcgtattggtagcgcacgttatattaccaaaaccaatgcaagcaccctggatacctttaaagcaaatgaagaaggttatctgggcgtcattattggcaatcgtatctattatcagaaccgcatcgacaaactgcataccacccgtagcgtttttgatgttcgtggtctgaccagcctgccgaaagtggatattctgtatggttatcaggatgatccggaatatctgtatgatgcagcaattcagcatggtgtgaaaggtattgtttatgcaggtatgggtgcgggtagcgttagcgttcgtggtattgccggtatgcgtaaagcaatggaaaaaggtgttgttgtgattcgtagcacccgtaccggtaatggtattgttccgcctgatgaagaactgcctggtctggttagcgatagcctgaatccggcacatgcacgtattctgctgatgctggcactgacccgtaccagcgatccgaaagttattcaagaatattttcatacctattaagctt

SEQ ID NO: 15 - protein, 40 aa, Synthetic construct
  REGION 1..40: note = PA(40) peptide
AAPAAPAPAAPAAPAPAAPAAAPAAPAPAAPAAPAPAAPA

SEQ ID NO: 16 - protein, 22 aa, Synthetic construct
  REGION 1..22: note = modified PA(20) peptide
  VARIANT 1: note = X = Pga (pyroglutamic acid)
  VARIANT 22: note = X = Ahx (6-aminohexanoic acid)
XAAPAAPAPAAPAAPAPAAPAX

SEQ ID NO: 17 - protein, 42 aa, Synthetic construct
  REGION 1..42: note = modified PA(40)-peptide
  VARIANT 1: note = X = Pga (pyroglutamic acid)
  VARIANT 42: note = X = Ahx (6-aminohexanoic acid)
XAAPAAPAPAAPAAPAPAAPAAAPAAPAPAAPAAPAPAAPAX